European Patent Application EP 4 570 256 A2, published June 18, 2025. Title: ENGINEERED T CELL RECEPTORS TARGETING EGFR ANTIGENS AND METHODS OF USE. Applicant: Board of Regents, The University of Texas System. The sequence listing filed with the application follows.

SEQUENCE LISTING (93 sequences)

SEQ ID NO: 1 - DNA, 1854 bp, Homo sapiens
  source 1..1854: mol_type = other DNA
atggatacctggctcgtatgctgggcaatttttagtctcttgaaagcaggactcacagaacctgaagtcacccagactcccagccatcaggtcacacagatgggacaggaagtgatcttgcgctgtgtccccatctctaatcacttatacttctattggtacagacaaatcttggggcagaaagtcgagtttctggtttccttttataataatgaaatctcagagaagtctgaaatattcgatgatcaattctcagttgaaaggcctgatggatcaaatttcactctgaagatccggtccacaaagctggaggactcagccatgtacttctgtgccagcagtggtgccgggggtaggtacgagcagtacttcgggccgggcaccaggctcacggtcacagaggacctgaaaaacgtgttcccacccgaggtcgctgtgtttgagccatcagaagcagagatctcccacacccaaaaggccacactggtatgcctggccacaggcttctaccccgaccacgtggagctgagctggtgggtgaatgggaaggaggtgcacagtggggtcagcacagacccgcagcccctcaaggagcagcccgccctcaatgactccagatactgcctgagcagccgcctgagggtctcggccaccttctggcagaacccccgcaaccacttccgctgtcaagtccagttctacgggctctcggagaatgacgagtggacccaggatagggccaaacccgtcacccagatcgtcagcgccgaggcctggggtagagcagactgtggcttcacctccgagtcttaccagcaaggggtcctgtctgccaccatcctctatgagatcttgctagggaaggccaccttgtatgccgtgctggtcagtgccctcgtgctgatggccatggtcaagagaaaggatttcagaggccgtgccaagcgaagcggatctggcgccacgaacttctctctgttaaagcaagcaggagatgttgaagaaaaccccgggcctatgtcactttctagcctgctgaaggtggtcacagcttcactgtggctaggacctggcattgcccagaagataactcaaacccaaccaggaatgttcgtgcaggaaaaggaggctgtgactctggactgcacatatgacaccagtgatccaagttatggtctattctggtacaagcagcccagcagtggggaaatgatttttcttatttatcaggggtcttatgaccagcaaaatgcaacagaaggtcgctactcattgaatttccagaaggcaagaaaatccgccaaccttgtcatctccgcttcacaactgggggactcagcaatgtacttctgtgcaatgagaggtatatctaactttggaaatgagaaattaacctttgggactggaacaagactcaccatcatacccaatatccagaagcctgaccctgccgtgtaccagctgagagactctaaatccagtgacaagtctgtctgcctattcaccgattttgattctcaaacaaatgtgtcacaaagtaaggattctgatgtgtatatcacagacaaaactgtgctagacatgaggtctatggacttcaagagcaacagtgctgtggcctggagcaacaaatctgactttgcatgtgcaaacgccttcaacaacagcattattccagcagacaccttcttccccagcccagaaagttcctgtgatgtcaagctggtcgagaaaagctttgaaacagatacgaacctaaactttcaaaacctgtcagtgattgtgttccgaatcctcctcctgaaagtggccgggtttaatctgctcatgacgctgcggctgtggtccagctga

SEQ ID NO: 2 - protein, 617 aa, Homo sapiens
MDTWLVCWAIFSLLKAGLTEPEVTQTPSHQVTQMGQEVILRCVPISNHLYFYWYRQILGQKVEFLVSFYNNEISEKSEIFDDQFSVERPDGSNFTLKIRSTKLEDSAMYFCASSGAGGRYEQYFGPGTRLTVTEDLKNVFPPEVAVFEPSEAEISHTQKATLVCLATGFYPDHVELSWWVNGKEVHSGVSTDPQPLKEQPALNDSRYCLSSRLRVSATFWQNPRNHFRCQVQFYGLSENDEWTQDRAKPVTQIVSAEAWGRADCGFTSESYQQGVLSATILYEILLGKATLYAVLVSALVLMAMVKRKDFRGRAKRSGSGATNFSLLKQAGDVEENPGPMSLSSLLKVVTASLWLGPGIAQKITQTQPGMFVQEKEAVTLDCTYDTSDPSYGLFWYKQPSSGEMIFLIYQGSYDQQNATEGRYSLNFQKARKSANLVISASQLGDSAMYFCAMRGISNFGNEKLTFGTGTRLTIIPNIQKPDPAVYQLRDSKSSDKSVCLFTDFDSQTNVSQSKDSDVYITDKTVLDMRSMDFKSNSAVAWSNKSDFACANAFNNSIIPADTFFPSPESSCDVKLVEKSFETDTNLNFQNLSVIVFRILLLKVAGFNLLMTLRLWSS

SEQ ID NO: 3 - protein, 320 aa, Homo sapiens
EPEVTQTPSHQVTQMGQEVILRCVPISNHLYFYWYRQILGQKVEFLVSFYNNEISEKSEIFDDQFSVERPDGSNFTLKIRSTKLEDSAMYFCASSGAGGRYEQYFGPGTRLTVTEDLKNVFPPEVAVFEPSEAEISHTQKATLVCLATGFYPDHVELSWWVNGKEVHSGVSTDPQPLKEQPALNDSRYCLSSRLRVSATFWQNPRNHFRCQVQFYGLSENDEWTQDRAKPVTQIVSAEAWGRADCGFTSESYQQGVLSATILYEILLGKATLYAVLVSALVLMAMVKRKDFRGRAKRSGSGATNFSLLKQAGDVEENPGP

SEQ ID NO: 4 - protein, 109 aa, Homo sapiens
EPEVTQTPSHQVTQMGQEVILRCVPISNHLYFYWYRQILGQKVEFLVSFYNNEISEKSEIFDDQFSVERPDGSNFTLKIRSTKLEDSAMYFCASSGAGGRYEQYFGPGT

SEQ ID NO: 5 - protein, 19 aa, Homo sapiens
MDTWLVCWAIFSLLKAGLT

SEQ ID NO: 6 - protein, 6 aa, Homo sapiens
SNHLYF

SEQ ID NO: 7 - protein, 5 aa, Homo sapiens
FYNNE

SEQ ID NO: 8 - protein, 12 aa, Homo sapiens
ASSGAGGRYEQY

SEQ ID NO: 9 - protein, 258 aa, Homo sapiens
AQKITQTQPGMFVQEKEAVTLDCTYDTSDPSYGLFWYKQPSSGEMIFLIYQGSYDQQNATEGRYSLNFQKARKSANLVISASQLGDSAMYFCAMRGISNFGNEKLTFGTGTRLTIIPNIQKPDPAVYQLRDSKSSDKSVCLFTDFDSQTNVSQSKDSDVYITDKTVLDMRSMDFKSNSAVAWSNKSDFACANAFNNSIIPADTFFPSPESSCDVKLVEKSFETDTNLNFQNLSVIVFRILLLKVAGFNLLMTLRLWSS

SEQ ID NO: 10 - protein, 117 aa, Homo sapiens
AQKITQTQPGMFVQEKEAVTLDCTYDTSDPSYGLFWYKQPSSGEMIFLIYQGSYDQQNATEGRYSLNFQKARKSANLVISASQLGDSAMYFCAMRGISNFGNEKLTFGTGTRLTIIP

SEQ ID NO: 11 - protein, 20 aa, Homo sapiens
MSLSSLLKVVTASLWLGPGI

SEQ ID NO: 12 - protein, 7 aa, Homo sapiens
TSDPSYG

SEQ ID NO: 13 - protein, 8 aa, Homo sapiens
QGSYDQQN

SEQ ID NO: 14 - protein, 14 aa, Homo sapiens
AMRGISNFGNEKLT

SEQ ID NO: 15 - DNA, 1865 bp, Homo sapiens
  source 1..1865: mol_type = other DNA
atgtcactttctagcctgctgaaggtggtcacagcttcactgtggctaggacctggcattgcccagaagataactcaaacccaaccaggaatgttcgtgcaggaaaaggaggctgtgactctggactgcacatatgacaccagtgatccaagttatggtctattctggtacaagcagcccagcagtggggaaatgatttttcttatttatcaggggtcttatgaccagcaaaatgcaacagaaggtcgctactcattgaatttccagaaggcaagaaaatccgccaaccttgtcatctccgcttcacaactgggggactcagcaatgtacttctgtgcaatgagagttatatctaactttggaaatgagaaattaacctttgggactggaacaagactcaccatcatacccaatatccagaagcctgaccctgccgtgtaccagctgagagactctaaatccagtgacaagtctgtctgcctattcaccgattttgattctcaaacaaatgtgtcacaaagtaaggattctgatgtgtatatcacagacaaaactgtgctagacatgaggtctatggacttcaagagcaacagtgctgtggcctggagcaacaaatctgactttgcatgtgcaaacgccttcaacaacagcattattccagcagacaccttcttccccagcccagaaagttcctgtgatgtcaagctggtcgagaaaagctttgaaacagatacgaacctaaactttcaaaacctgtcagtgattgggttccgaatcctcctcctgaaagtggccgggttttatctgctcatgacgctgcggctgtggtccagcgtcgacgtgccaagcgaagcggatctggcgccacgaacttctctctgttaaagcaagcaggagatgttgaagaaaaccccgggcctctcgagatggatacctggctcgtatgctgggcaatttttagtctcttgaaagcaggactcacagaacctgaagtcacccagactcccagccatcaggtcacacagatgggacaggaagtgatcttgcgctgtgtccccatctctaatcacttatacttctattggtacagacaaatcttggggcagaaagtcgagtttctggtttccttttataataatgaaatctcagagaagtctgaaatattcgatgatcaattctcagttgaaaggcctgatggatcaaatttcactctgaagatccggtccacaaagctggaggactcagccatgtacttctgtgccagcagtctcggcgggggcacctacgagcagtacttcgggccgggcaccaggctcacggtcacagaggacctgaaaaacgtgttcccacccgaggtcgctgtgtttgagccatcagaagcagagatctcccacacccaaaaggccacactggtgtgcctggccacaggcttcttccctgaccacgtggagctgagctggtgggtgaatgggaaggaggtgcacagtggggtcagcacagacccgcagcccctcaaggagcagcccgccctcaatgactccagatactgcctgagcagccgcctgagggtctcggccaccttctggcagaacccccgcaaccacttccgctgtcaagtccagttctacgggctctcggagaatgacgagtggacccaggatagggccaaacctgtcacccagatcgtcagcgccgaggcctggggtagagcagactgtggcttcacctccgagtcttaccagcaaggggtcctgtctgccaccatcctctatgagatcttgctagggaaggccaccttgtatgccgtgctggtcagtgccctcgtgctgatggccatggtcaagagaaaggattccagaggctag

SEQ ID NO: 16 - protein, 621 aa, Homo sapiens
MSLSSLLKVVTASLWLGPGIAQKITQTQPGMFVQEKEAVTLDCTYDTSDPSYGLFWYKQPSSGEMIFLIYQGSYDQQNATEGRYSLNFQKARKSANLVISASQLGDSAMYFCAMRVISNFGNEKLTFGTGTRLTIIPNIQKPDPAVYQLRDSKSSDKSVCLFTDFDSQTNVSQSKDSDVYITDKTVLDMRSMDFKSNSAVAWSNKSDFACANAFNNSIIPADTFFPSPESSCDVKLVEKSFETDTNLNFQNLSVIGFRILLLKVAGFYLLMTLRLWSSVDRAKRSGSGATNFSLLKQAGDVEENPGPLEMDTWLVCWAIFSLLKAGLTEPEVTQTPSHQVTQMGQEVILRCVPISNHLYFYWYRQILGQKVEFLVSFYNNEISEKSEIFDDQFSVERPDGSNFTLKIRSTKLEDSAMYFCASSLGGGTYEQYFGPGTRLTVTEDLKNVFPPEVAVFEPSEAEISHTQKATLVCLATGFFPDHVELSWWVNGKEVHSGVSTDPQPLKEQPALNDSRYCLSSRLRVSATFWQNPRNHFRCQVQFYGLSENDEWTQDRAKPVTQIVSAEAWGRADCGFTSESYQQGVLSATILYEILLGKATLYAVLVSALVLMAMVKRKDSRG

SEQ ID NO: 17 - protein, 289 aa, Homo sapiens
AQKITQTQPGMFVQEKEAVTLDCTYDTSDPSYGLFWYKQPSSGEMIFLIYQGSYDQQNATEGRYSLNFQKARKSANLVISASQLGDSAMYFCAMRVISNFGNEKLTFGTGTRLTIIPNIQKPDPAVYQLRDSKSSDKSVCLFTDFDSQTNVSQSKDSDVYITDKTVLDMRSMDFKSNSAVAWSNKSDFACANAFNNSIIPADTFFPSPESSCDVKLVEKSFETDTNLNFQNLSVIGFRILLLKVAGFYLLMTLRLWSSVDRAKRSGSGATNFSLLKQAGDVEENPGPLE

SEQ ID NO: 18 - protein, 117 aa, Homo sapiens
AQKITQTQPGMFVQEKEAVTLDCTYDTSDPSYGLFWYKQPSSGEMIFLIYQGSYDQQNATEGRYSLNFQKARKSANLVISASQLGDSAMYFCAMRVISNFGNEKLTFGTGTRLTIIP

SEQ ID NO: 19 - protein, 20 aa, Homo sapiens
MSLSSLLKVVTASLWLGPGI

SEQ ID NO: 20 - protein, 7 aa, Homo sapiens
TSDPSYG

SEQ ID NO: 21 - protein, 8 aa, Homo sapiens
QGSYDQQN

SEQ ID NO: 22 - protein, 14 aa, Homo sapiens
AMRVISNFGNEKLT

SEQ ID NO: 23 - protein, 293 aa, Homo sapiens
EPEVTQTPSHQVTQMGQEVILRCVPISNHLYFYWYRQILGQKVEFLVSFYNNEISEKSEIFDDQFSVERPDGSNFTLKIRSTKLEDSAMYFCASSLGGGTYEQYFGPGTRLTVTEDLKNVFPPEVAVFEPSEAEISHTQKATLVCLATGFFPDHVELSWWVNGKEVHSGVSTDPQPLKEQPALNDSRYCLSSRLRVSATFWQNPRNHFRCQVQFYGLSENDEWTQDRAKPVTQIVSAEAWGRADCGFTSESYQQGVLSATILYEILLGKATLYAVLVSALVLMAMVKRKDSRG

SEQ ID NO: 24 - protein, 114 aa, Homo sapiens
EPEVTQTPSHQVTQMGQEVILRCVPISNHLYFYWYRQILGQKVEFLVSFYNNEISEKSEIFDDQFSVERPDGSNFTLKIRSTKLEDSAMYFCASSLGGGTYEQYFGPGTRLTVT

SEQ ID NO: 25 - protein, 19 aa, Homo sapiens
MDTWLVCWAIFSLLKAGLT

SEQ ID NO: 26 - protein, 5 aa, Homo sapiens
SNHLY

SEQ ID NO: 27 - protein, 6 aa, Homo sapiens
FYNNEI

SEQ ID NO: 28 - protein, 13 aa, Homo sapiens
ASSLGGGTYEQYF

SEQ ID NO: 29 - DNA, 1842 bp, Homo sapiens
  source 1..1842: mol_type = other DNA
atgctgttctccagcctgctgtgtgtatttgtggccttcagctactctggatcaagtgtggcccagaaggttactcaagcccagtcatcagtatccatgccagtgaggaaagcagtcaccctgaactgcctgtatgaaacaagttggtggtcatattatattttttggtacaagcaacttcccagcaaagagatgattttccttattcgccagggttctgatgaacagaatgcaaaaagtggtcgctattctgtcaacttcaagaaagcagcgaaatccgtcgccttaaccatttcagccttacagctagaagattcagcaaagtacttttgtgctcttggggatagcaactatcagttaatctggggcgctgggaccaagctaattataaagccagatatccagaaccctgaccctgccgtgtaccagctgagagactctaaatccagtgacaagtctgtctgcctattcaccgattttgattctcaaacaaatgtgtcacaaagtaaggattctgatgtgtatatcacagacaaatgcgtgctagacatgaggtctatggacttcaagagcaacagtgctgtggcctggagcaacaaatctgactttgcatgtgcaaacgccttcaacaacagcattattccagaagacaccttcttccccagcccagaaagttcctgtgatgtcaagctggtcgagaaaagctttgaaacagatacgaacctaaactttcaaaacctgtcagtgattgggttccgaatcctcctcctgaaagtggccgggtttaatctgctcatgacgctgcggctgtggtccagccgtgccaagcgaagcggatctggcgccacgaacttctctctgttaaagcaagcaggagatgttgaagaaaaccccgggcctatggactcctggaccttctgctgtgtgtccctttgcatcctggtagcgaagcatacagatgctggagttatccagtcaccccgccatgaggtgacagagatgggacaagaagtgactctgagatgtaaaccaatttcaggccacaactcccttttctggtacagacagaccatgatgcggggactggagttgctcatttactttaacaacaacgttccgatagatgattcagggatgcccgaggatcgattctcagctaagatgcctaatgcatcattctccactctgaagatccagccctcagaacccagggactcagctgtgtacttctgtgccagcagagccgggacaggggaggtcaatgagcagttcttcgggccagggacacggctcaccgtgctagaggacctgaaaaacgtgttcccacccgaggtcgctgtgtttgagccatcagaagcagagatctcccacacccaaaaggccacactggtgtgcctggccacaggcttctaccccgaccacgtggagctgagctggtgggtgaatgggaaggaggtgcacagtggggtctgcacagacccgcagcccctcaaggagcagcccgccctcaatgactccagatactgcctgagcagccgcctgagggtctcggccaccttctggcagaacccccgcaaccacttccgctgtcaagtccagttctacgggctctcggagaatgacgagtggacccaggatagggccaaacctgtcacccagatcgtcagcgccgaggcctggggtagagcagactgtggcttcacctccgagtcttaccagcaaggggtcctgtctgccaccatcctctatgagatcttgctagggaaggccaccttgtatgccgtgctggtcagtgccctcgtgctgatggccatggtcaagagaaaggattccagaggctaa

SEQ ID NO: 30 - protein, 613 aa, Homo sapiens
MLFSSLLCVFVAFSYSGSSVAQKVTQAQSSVSMPVRKAVTLNCLYETSWWSYYIFWYKQLPSKEMIFLIRQGSDEQNAKSGRYSVNFKKAAKSVALTISALQLEDSAKYFCALGDSNYQLIWGAGTKLIIKPDIQNPDPAVYQLRDSKSSDKSVCLFTDFDSQTNVSQSKDSDVYITDKCVLDMRSMDFKSNSAVAWSNKSDFACANAFNNSIIPEDTFFPSPESSCDVKLVEKSFETDTNLNFQNLSVIGFRILLLKVAGFNLLMTLRLWSSRAKRSGSGATNFSLLKQAGDVEENPGPMDSWTFCCVSLCILVAKHTDAGVIQSPRHEVTEMGQEVTLRCKPISGHNSLFWYRQTMMRGLELLIYFNNNVPIDDSGMPEDRFSAKMPNASFSTLKIQPSEPRDSAVYFCASRAGTGEVNEQFFGPGTRLTVLEDLKNVFPPEVAVFEPSEAEISHTQKATLVCLATGFYPDHVELSWWVNGKEVHSGVCTDPQPLKEQPALNDSRYCLSSRLRVSATFWQNPRNHFRCQVQFYGLSENDEWTQDRAKPVTQIVSAEAWGRADCGFTSESYQQGVLSATILYEILLGKATLYAVLVSALVLMAMVKRKDSRG

SEQ ID NO: 31 - protein, 279 aa, Homo sapiens
QKVTQAQSSVSMPVRKAVTLNCLYETSWWSYYIFWYKQLPSKEMIFLIRQGSDEQNAKSGRYSVNFKKAAKSVALTISALQLEDSAKYFCALGDSNYQLIWGAGTKLIIKPDIQNPDPAVYQLRDSKSSDKSVCLFTDFDSQTNVSQSKDSDVYITDKCVLDMRSMDFKSNSAVAWSNKSDFACANAFNNSIIPEDTFFPSPESSCDVKLVEKSFETDTNLNFQNLSVIGFRILLLKVAGFNLLMTLRLWSSRAKRSGSGATNFSLLKQAGDVEENPGP

SEQ ID NO: 32 - protein, 112 aa, Homo sapiens
QKVTQAQSSVSMPVRKAVTLNCLYETSWWSYYIFWYKQLPSKEMIFLIRQGSDEQNAKSGRYSVNFKKAAKSVALTISALQLEDSAKYFCALGDSNYQLIWGAGTKLIIKPD

SEQ ID NO: 33 - protein, 21 aa, Homo sapiens
MLFSSLLCVFVAFSYSGSSVA

SEQ ID NO: 34 - protein, 7 aa, Homo sapiens
TSWWSYY

SEQ ID NO: 35 - protein, 8 aa, Homo sapiens
QGSDEQNA

SEQ ID NO: 36 - protein, 9 aa, Homo sapiens
LGDSNYQLI

SEQ ID NO: 37 - protein, 292 aa, Homo sapiens
GVIQSPRHEVTEMGQEVTLRCKPISGHNSLFWYRQTMMRGLELLIYFNNNVPIDDSGMPEDRFSAKMPNASFSTLKIQPSEPRDSAVYFCASRAGTGEVNEQFFGPGTRLTVLEDLKNVFPPEVAVFEPSEAEISHTQKATLVCLATGFYPDHVELSWWVNGKEVHSGVCTDPQPLKEQPALNDSRYCLSSRLRVSATFWQNPRNHFRCQVQFYGLSENDEWTQDRAKPVTQIVSAEAWGRADCGFTSESYQQGVLSATILYEILLGKATLYAVLVSALVLMAMVKRKDSRG

SEQ ID NO: 38 - protein, 113 aa, Homo sapiens
GVIQSPRHEVTEMGQEVTLRCKPISGHNSLFWYRQTMMRGLELLIYFNNNVPIDDSGMPEDRFSAKMPNASFSTLKIQPSEPRDSAVYFCASRAGTGEVNEQFFGPGTRLTVL

SEQ ID NO: 39 - protein, 21 aa, Homo sapiens
MDSWTFCCVSLCILVAKHTDA

SEQ ID NO: 40 - protein, 5 aa, Homo sapiens
SGHNS

SEQ ID NO: 41 - protein, 6 aa, Homo sapiens
FNNNVP

SEQ ID NO: 42 - protein, 13 aa, Homo sapiens
ASRAGTGEVNEQF

SEQ ID NO: 43 - DNA, 1854 bp, Homo sapiens
  source 1..1854: mol_type = other DNA
atgtcactttctagcctgctgaaggtggtcacagcttcactgtggctaggacctggcattgcccagaagataactcaaacccaaccaggaatgttcgtgcaggaaaaggaggctgtgactctggactgcacatatgacaccagtgatcaaagttatggtctattctggtacaagcagcccagcagtggggaaatgatttttcttatttatcaggggtcttatgacgagcaaaatgcaacagaaggtcgctactcattgaatttccagaaggcaagaaaatccgccaaccttgtcatctccgcttcacaactgggggactcagcaatgtatttctgtgcaatgagagaggtctttggaaatgagaaattaacctttgggactggaacaagactcaccatcatacccaatatccagaaccctgaccctgccgtgtaccagctgagagactctaaatccagtgacaagtctgtctgcctattcaccgattttgattctcaaacaaatgtgtcacaaagtaaggattctgatgtgtatatcacagacaaatgcgtgctagacatgaggtctatggacttcaagagcaacagtgctgtggcctggagcaacaaatctgactttgcatgtgcaaacgccttcaacaacagcattattccagaagacaccttcttccccagcccagaaagttcctgtgatgtcaagctggtcgagaaaagctttgaaacagatacgaacctaaactttcaaaacctgtcagtgattgggttccgaatcctcctcctgaaagtggccgggtttaatctgctcatgacgctgcggctgtggtccagccgtgccaagcgaagcggatctggcgccacgaacttctctctgttaaagcaagcaggagatgttgaagaaaaccccgggcctatgagcccaatattcacctgcatcacaatcctttgtctgctggctgcaggttctcctggtgaagaagtcgcccagactccaaaacatcttgtcagaggggaaggacagaaagcaaaattatattgtgccccaataaaaggacacagttatgttttttggtaccaacaggtcctgaaaaacgagttcaagttcttgatttccttccagaatgaaaatgtctttgatgaaacaggtatgcccaaggaaagattttcagctaagtgcctcccaaattcaccctgtagccttgagatccaggctacgaagcttgaggattcagcagtgtatttttgtgccagcagccctcctccctcaaacacctacaatgagcagttcttcgggccagggacacggctcaccgtgctagaggacctgaaaaacgtgttcccacccgaggtcgctgtgtttgagccatcagaagcagagatctcccacacccaaaaggccacactggtgtgcctggccacaggcttctaccccgaccacgtggagctgagctggtgggtgaatgggaaggaggtgcacagtggggtctgcacagacccgcagcccctcaaggagcagcccgccctcaatgactccagatactgcctgagcagccgcctgagggtctcggccaccttctggcagaacccccgcaaccacttccgctgtcaagtccagttctacgggctctcggagaatgacgagtggacccaggatagggccaaacctgtcacccagatcgtcagcgccgaggcctggggtagagcagactgtggcttcacctccgagtcttaccagcaaggggtcctgtctgccaccatcctctatgagatcttgctagggaaggccaccttgtatgccgtgctggtcagtgccctcgtgctgatggccatggtcaagagaaaggattccagaggctaa

SEQ ID NO: 44 - protein, 617 aa, Homo sapiens
MSLSSLLKVVTASLWLGPGIAQKITQTQPGMFVQEKEAVTLDCTYDTSDQSYGLFWYKQPSSGEMIFLIYQGSYDEQNATEGRYSLNFQKARKSANLVISASQLGDSAMYFCAMREVFGNEKLTFGTGTRLTIIPNIQNPDPAVYQLRDSKSSDKSVCLFTDFDSQTNVSQSKDSDVYITDKCVLDMRSMDFKSNSAVAWSNKSDFACANAFNNSIIPEDTFFPSPESSCDVKLVEKSFETDTNLNFQNLSVIGFRILLLKVAGFNLLMTLRLWSSRAKRSGSGATNFSLLKQAGDVEENPGPMSPIFTCITILCLLAAGSPGEEVAQTPKHLVRGEGQKAKLYCAPIKGHSYVFWYQQVLKNEFKFLISFQNENVFDETGMPKERFSAKCLPNSPCSLEIQATKLEDSAVYFCASSPPPSNTYNEQFFGPGTRLTVLEDLKNVFPPEVAVFEPSEAEISHTQKATLVCLATGFYPDHVELSWWVNGKEVHSGVCTDPQPLKEQPALNDSRYCLSSRLRVSATFWQNPRNHFRCQVQFYGLSENDEWTQDRAKPVTQIVSAEAWGRADCGFTSESYQQGVLSATILYEILLGKATLYAVLVSALVLMAMVKRKDSRG

SEQ ID NO: 45 - protein, 282 aa, Homo sapiens
QKITQTQPGMFVQEKEAVTLDCTYDTSDQSYGLFWYKQPSSGEMIFLIYQGSYDEQNATEGRYSLNFQKARKSANLVISASQLGDSAMYFCAMREVFGNEKLTFGTGTRLTIIPNIQNPDPAVYQLRDSKSSDKSVCLFTDFDSQTNVSQSKDSDVYITDKCVLDMRSMDFKSNSAVAWSNKSDFACANAFNNSIIPEDTFFPSPESSCDVKLVEKSFETDTNLNFQNLSVIGFRILLLKVAGFNLLMTLRLWSSRAKRSGSGATNFSLLKQAGDVEENPGP

SEQ ID NO: 46 - protein, 114 aa, Homo sapiens
QKITQTQPGMFVQEKEAVTLDCTYDTSDQSYGLFWYKQPSSGEMIFLIYQGSYDEQNATEGRYSLNFQKARKSANLVISASQLGDSAMYFCAMREVFGNEKLTFGTGTRLTIIP

SEQ ID NO: 47 - protein, 21 aa, Homo sapiens
MSLSSLLKVVTASLWLGPGIA

SEQ ID NO: 48 - protein, 7 aa, Homo sapiens
TSDQSYG

SEQ ID NO: 49 - protein, 8 aa, Homo sapiens
QGSYDEQN

SEQ ID NO: 50 - protein, 12 aa, Homo sapiens
AMREVFGNEKLT

SEQ ID NO: 51 - protein, 294 aa, Homo sapiens
EEVAQTPKHLVRGEGQKAKLYCAPIKGHSYVFWYQQVLKNEFKFLISFQNENVFDETGMPKERFSAKCLPNSPCSLEIQATKLEDSAVYFCASSPPPSNTYNEQFFGPGTRLTVLEDLKNVFPPEVAVFEPSEAEISHTQKATLVCLATGFYPDHVELSWWVNGKEVHSGVCTDPQPLKEQPALNDSRYCLSSRLRVSATFWQNPRNHFRCQVQFYGLSENDEWTQDRAKPVTQIVSAEAWGRADCGFTSESYQQGVLSATILYEILLGKATLYAVLVSALVLMAMVKRKDSRG

SEQ ID NO: 52 - protein, 115 aa, Homo sapiens
EEVAQTPKHLVRGEGQKAKLYCAPIKGHSYVFWYQQVLKNEFKFLISFQNENVFDETGMPKERFSAKCLPNSPCSLEIQATKLEDSAVYFCASSPPPSNTYNEQFFGPGTRLTVL

SEQ ID NO: 53 - protein, 20 aa, Homo sapiens
MSPIFTCITILCLLAAGSPG

SEQ ID NO: 54 - protein, 5 aa, Homo sapiens
KGHSY

SEQ ID NO: 55 - protein, 6 aa, Homo sapiens
FQNENV

SEQ ID NO: 56 - protein, 14 aa, Homo sapiens
ASSPPPSNTYNEQF

SEQ ID NO: 57 - DNA, 1854 bp, Homo sapiens
  source 1..1854: mol_type = other DNA
atgtcactttctagcctgctgaaggtggtcacagcttcactgtggctaggacctggcattgcccagaagataactcaaacccaaccaggaatgttcgtgcaggaaaaggaggctgtgactctggactgcacatatgacaccagtgatcaaagttatggtctattctggtacaagcagcccagcagtggggaaatgatttttcttatttatcaggggtcttatgacgagcaaaatgcaacagaaggtcgctactcattgaatttccagaaggcaagaaaatccgccaaccttgtcatctccgcttcacaactgggggactcagcaatgtatttctgtgcaatgagagaggtctttggaaatgagaaattaacctttgggactggaacaagactcaccatcatacccaatatccagaaccctgaccctgccgtgtaccagctgagagactctaaatccagtgacaagtctgtctgcctattcaccgattttgattctcaaacaaatgtgtcacaaagtaaggattctgatgtgtatatcacagacaaatgcgtgctagacatgaggtctatggacttcaagagcaacagtgctgtggcctggagcaacaaatctgactttgcatgtgcaaacgccttcaacaacagcattattccagaagacaccttcttccccagcccagaaagttcctgtgatgtcaagctggtcgagaaaagctttgaaacagatacgaacctaaactttcaaaacctgtcagtgattgggttccgaatcctcctcctgaaagtggccgggtttaatctgctcatgacgctgcggctgtggtccagccgtgccaagcgaagcggatctggcgccacgaacttctctctgttaaagcaagcaggagatgttgaagaaaaccccgggcctatgagcccaatattcacctgcatcacaatcctttgtctgctggctgcaggttctcctggtgaagaagtcgcccagactccaaaacatcttgtcagaggggaaggacagaaagcaaaattatattgtgccccaataaaaggacacagttatgttttttggtaccaacaggtcctgaaaaacgagttcaagttcttgatttccttccagaatgaaaatgtctttgatgaaacaggtatgcccaagggaagattttcagctaagtgcctcccaaattcaccctgtagccttgagatccaggctacgaagcttgaggattcagcagtgtatttttgtgccagcagccatagaagttggaaggggggtgatacgcagccccagcattttggtgatgggactcgactctccatcctagaggacctgaacaaggtgttcccacccgaggtcgctgtgtttgagccatcagaagcagagatctcccacacccaaaaggccacactggtgtgcctggccacaggcttcttccctgaccacgtggagctgagctggtgggtgaatgggaaggaggtgcacagtggggtctgcacggacccgcagcccctcaaggagcagcccgccctcaatgactccagatactgcctgagcagccgcctgagggtctcggccaccttctggcagaacccccgcaaccacttccgctgtcaagtccagttctacgggctctcggagaatgacgagtggacccaggatagggccaaacccgtcacccagatcgtcagcgccgaggcctggggtagagcagactgtggctttacctcggtgtcctaccagcaaggggtcctgtctgccaccatcctctatgagatcctgctagggaaggccaccctgtatgctgtgctggtcagcgcccttgtgttgatggccatggtcaagagaaaggatttctga

SEQ ID NO: 58 - protein, 617 aa, Homo sapiens
MSLSSLLKVVTASLWLGPGIAQKITQTQPGMFVQEKEAVTLDCTYDTSDQSYGLFWYKQPSSGEMIFLIYQGSYDEQNATEGRYSLNFQKARKSANLVISASQLGDSAMYFCAMREVFGNEKLTFGTGTRLTIIPNIQNPDPAVYQLRDSKSSDKSVCLFTDFDSQTNVSQSKDSDVYITDKCVLDMRSMDFKSNSAVAWSNKSDFACANAFNNSIIPEDTFFPSPESSCDVKLVEKSFETDTNLNFQNLSVIGFRILLLKVAGFNLLMTLRLWSSRAKRSGSGATNFSLLKQAGDVEENPGPMSPIFTCITILCLLAAGSPGEEVAQTPKHLVRGEGQKAKLYCAPIKGHSYVFWYQQVLKNEFKFLISFQNENVFDETGMPKGRFSAKCLPNSPCSLEIQATKLEDSAVYFCASSHRSWKGGDTQPQHFGDGTRLSILEDLNKVFPPEVAVFEPSEAEISHTQKATLVCLATGFFPDHVELSWWVNGKEVHSGVCTDPQPLKEQPALNDSRYCLSSRLRVSATFWQNPRNHFRCQVQFYGLSENDEWTQDRAKPVTQIVSAEAWGRADCGFTSVSYQQGVLSATILYEILLGKATLYAVLVSALVLMAMVKRKDF

SEQ ID NO: 59 - protein, 283 aa, Homo sapiens
AQKITQTQPGMFVQEKEAVTLDCTYDTSDQSYGLFWYKQPSSGEMIFLIYQGSYDEQNATEGRYSLNFQKARKSANLVISASQLGDSAMYFCAMREVFGNEKLTFGTGTRLTIIPNIQNPDPAVYQLRDSKSSDKSVCLFTDFDSQTNVSQSKDSDVYITDKCVLDMRSMDFKSNSAVAWSNKSDFACANAFNNSIIPEDTFFPSPESSCDVKLVEKSFETDTNLNFQNLSVIGFRILLLKVAGFNLLMTLRLWSSRAKRSGSGATNFSLLKQAGDVEENPGP

SEQ ID NO: 60 - protein, 115 aa, Homo sapiens
AQKITQTQPGMFVQEKEAVTLDCTYDTSDQSYGLFWYKQPSSGEMIFLIYQGSYDEQNATEGRYSLNFQKARKSANLVISASQLGDSAMYFCAMREVFGNEKLTFGTGTRLTIIP

SEQ ID NO: 61 - protein, 20 aa, Homo sapiens
MSLSSLLKVVTASLWLGPGI

SEQ ID NO: 62 - protein, 7 aa, Homo sapiens
TSDQSYG

SEQ ID NO: 63 - protein, 8 aa, Homo sapiens
QGSYDEQN

SEQ ID NO: 64 - protein, 12 aa, Homo sapiens
AMREVFGNEKLT

SEQ ID NO: 65 - protein, 294 aa, Homo sapiens
EEVAQTPKHLVRGEGQKAKLYCAPIKGHSYVFWYQQVLKNEFKFLISFQNENVFDETGMPKGRFSAKCLPNSPCSLEIQATKLEDSAVYFCASSHRSWKGGDTQPQHFGDGTRLSILEDLNKVFPPEVAVFEPSEAEISHTQKATLVCLATGFFPDHVELSWWVNGKEVHSGVCTDPQPLKEQPALNDSRYCLSSRLRVSATFWQNPRNHFRCQVQFYGLSENDEWTQDRAKPVTQIVSAEAWGRADCGFTSVSYQQGVLSATILYEILLGKATLYAVLVSALVLMAMVKRKDF

SEQ ID NO: 66 - protein, 117 aa, Homo sapiens
EEVAQTPKHLVRGEGQKAKLYCAPIKGHSYVFWYQQVLKNEFKFLISFQNENVFDETGMPKGRFSAKCLPNSPCSLEIQATKLEDSAVYFCASSHRSWKGGDTQPQHFGDGTRLSIL

SEQ ID NO: 67 - protein, 20 aa, Homo sapiens
MSPIFTCITILCLLAAGSPG

SEQ ID NO: 68 - protein, 5 aa, Homo sapiens
KGHSY

SEQ ID NO: 69 - protein, 6 aa, Homo sapiens
FQNENV

SEQ ID NO: 70 - protein, 16 aa, Homo sapiens
ASSHRSWKGGDTQPQH

SEQ ID NO: 71 - DNA, 1866 bp, Homo sapiens
  source 1..1866: mol_type = other DNA
atgtcactttctagcctgctgaaggtggtcacagcttcactgtggctaggacctggcattgcccagaagataactcaaacccaaccaggaatgttcgtgcaggaaaaggaggctgtgactctggactgcacatatgacaccagtgatccaagttatggtctattctggtacaagcagcccagcagtggggaaatgatttttcttatttatcaggggtcttatgaccagcaaaatgcaacagaaggtcgctactcattgaatttccagaaggcaagaaaatccgccaaccttgtcatctccgcttcacaactgggggactcagcaatgtacttctgtgcaatgaggagtgggcatctgtctaactttggaaatgagaaattaacctttgggactggaacaagactcaccatcatacccaatatccagaaccctgaccctgccgtgtaccagctgagagactctaaatccagtgacaagtctgtctgcctattcaccgattttgattctcaaacaaatgtgtcacaaagtaaggattctgatgtgtatatcacagacaaatgcgtgctagacatgaggtctatggacttcaagagcaacagtgctgtggcctggagcaacaaatctgactttgcatgtgcaaacgccttcaacaacagcattattccagaagacaccttcttccccagcccagaaagttcctgtgatgtcaagctggtcgagaaaagctttgaaacagatacgaacctaaactttcaaaacctgtcagtgattgggttccgaatcctcctcctgaaagtggccgggtttaatctgctcatgacgctgcggctgtggtccagccgtgccaagcgaagcggatctggcgccacgaacttctctctgttaaagcaagcaggagatgttgaagaaaaccccgggcctatgagcccaatattcacctgcatcacaatcctttgtctgctggctgcaggttctcctggtgaagaagtcgcccagactccaaaacatcttgtcagaggggaaggacagaaagcaaaattatattgtgccccaataaaaggacacagttatgttttttggtaccaacaggtcctgaaaaacgagttcaagttcttgatttccttccagaatgaaaatgtctttgatgaaacaggtatgcccaagggaagattttcagctaagtgcctcccaaattcaccctgtagccttgagatccaggctacgaagcttgaggattcagcagtgtatttttgtgccagcagccatagaagttggaaggggggtgatacgcagccccagcattttggtgatgggactcgactctccatcctagaggacctgaacaaggtgttcccacccgaggtcgctgtgtttgagccatcagaagcagagatctcccacacccaaaaggccacactggtgtgcctggccacaggcttcttccctgaccacgtggagctgagctggtgggtgaatgggaaggaggtgcacagtggggtctgcacggacccgcagcccctcaaggagcagcccgccctcaatgactccagatactgcctgagcagccgcctgagggtctcggccaccttctggcagaacccccgcaaccacttccgctgtcaagtccagttctacgggctctcggagaatgacgagtggacccaggatagggccaaacccgtcacccagatcgtcagcgccgaggcctggggtagagcagactgtggctttacctcggtgtcctaccagcaaggggtcctgtctgccaccatcctctatgagatcctgctagggaaggccaccctgtatgctgtgctggtcagcgcccttgtgttgatggccatggtcaagagaaaggatttctga

SEQ ID NO: 72 - protein, 621 aa, Homo sapiens
MSLSSLLKVVTASLWLGPGIAQKITQTQPGMFVQEKEAVTLDCTYDTSDPSYGLFWYKQPSSGEMIFLIYQGSYDQQNATEGRYSLNFQKARKSANLVISASQLGDSAMYFCAMRSGHLSNFGNEKLTFGTGTRLTIIPNIQNPDPAVYQLRDSKSSDKSVCLFTDFDSQTNVSQSKDSDVYITDKCVLDMRSMDFKSNSAVAWSNKSDFACANAFNNSIIPEDTFFPSPESSCDVKLVEKSFETDTNLNFQNLSVIGFRILLLKVAGFNLLMTLRLWSSRAKRSGSGATNFSLLKQAGDVEENPGPMSPIFTCITILCLLAAGSPGEEVAQTPKHLVRGEGQKAKLYCAPIKGHSYVFWYQQVLKNEFKFLISFQNENVFDETGMPKGRFSAKCLPNSPCSLEIQATKLEDSAVYFCASSHRSWKGGDTQPQHFGDGTRLSILEDLNKVFPPEVAVFEPSEAEISHTQKATLVCLATGFFPDHVELSWWVNGKEVHSGVCTDPQPLKEQPALNDSRYCLSSRLRVSATFWQNPRNHFRCQVQFYGLSENDEWTQDRAKPVTQIVSAEAWGRADCGFTSVSYQQGVLSATILYEILLGKATLYAVLVSALVLMAMVKRKDF

SEQ ID NO: 73 - protein, 287 aa, Homo sapiens
AQKITQTQPGMFVQEKEAVTLDCTYDTSDPSYGLFWYKQPSSGEMIFLIYQGSYDQQNATEGRYSLNFQKARKSANLVISASQLGDSAMYFCAMRSGHLSNFGNEKLTFGTGTRLTIIPNIQNPDPAVYQLRDSKSSDKSVCLFTDFDSQTNVSQSKDSDVYITDKCVLDMRSMDFKSNSAVAWSNKSDFACANAFNNSIIPEDTFFPSPESSCDVKLVEKSFETDTNLNFQNLSVIGFRILLLKVAGFNLLMTLRLWSSRAKRSGSGATNFSLLKQAGDVEENPGP

SEQ ID NO: 74 - protein, 119 aa, Homo sapiens
AQKITQTQPGMFVQEKEAVTLDCTYDTSDPSYGLFWYKQPSSGEMIFLIYQGSYDQQNATEGRYSLNFQKARKSANLVISASQLGDSAMYFCAMRSGHLSNFGNEKLTFGTGTRLTIIP

SEQ ID NO: 75 - protein, 20 aa, Homo sapiens
MSLSSLLKVVTASLWLGPGI

SEQ ID NO: 76 - protein, 7 aa, Homo sapiens
TSDPSYG

SEQ ID NO: 77 - protein, 8 aa, Homo sapiens
QGSYDQQN

SEQ ID NO: 78 - protein, 16 aa, Homo sapiens
AMRSGHLSNFGNEKLT

SEQ ID NO: 79 - protein, 294 aa, Homo sapiens; identical to SEQ ID NO: 65

SEQ ID NO: 80 - protein, 117 aa, Homo sapiens; identical to SEQ ID NO: 66

SEQ ID NO: 81 - protein, 20 aa, Homo sapiens
MSPIFTCITILCLLAAGSPG

SEQ ID NO: 82 - protein, 5 aa, Homo sapiens
KGHSY

SEQ ID NO: 83 - protein, 6 aa, Homo sapiens
FQNENV

SEQ ID NO: 84 - protein, 16 aa, Homo sapiens
ASSHRSWKGGDTQPQH

SEQ ID NO: 85 - protein, 9 aa, synthetic construct
  REGION 1..9: note = synthetic polypeptide
HVKITDFGR

SEQ ID NO: 86 - protein, 5 aa, synthetic construct
  REGION 1..5: note = synthetic polypeptide
GSGGS

SEQ ID NO: 87 - protein, 4 aa, synthetic construct
  REGION 1..4: note = synthetic polypeptide
GGGS

SEQ ID NO: 88 - protein, 4 aa, synthetic construct
  REGION 1..4: note = synthetic polypeptide
GGSG

SEQ ID NO: 89 - protein, 5 aa, synthetic construct
  REGION 1..5: note = synthetic polypeptide
GGSGG

SEQ ID NO: 90 - protein, 5 aa, synthetic construct
  REGION 1..5: note = synthetic polypeptide
GSGSG

SEQ ID NO: 91 - protein, 5 aa, synthetic construct
  REGION 1..5: note = synthetic polypeptide
GSGGG

SEQ ID NO: 92 - protein, 5 aa, synthetic construct
  REGION 1..5: note = synthetic polypeptide
GGGSG

SEQ ID NO: 93 - protein, 5 aa, synthetic construct
  REGION 1..5: note = synthetic polypeptide
GSSSG